European Patent Application EP 4 403 627 A2, published July 24, 2024. Title: PRODUCTION OF CAROTENOIDS AND APOCAROTENOIDS. Applicant: Agency for Science, Technology and Research. Application EP. The sequence listing filed with the application follows.

SEQUENCE LISTING (4 sequences)

SEQ ID NO: 1 - DNA, 32 bp, Bacteriophage T7
  source 1..32: mol_type = unassigned DNA
taatacgactcactataggggaattgtgagcg

SEQ ID NO: 2 - DNA, 32 bp, synthetic construct
  misc_feature 1..32: note = TM1 promoter
  source 1..32: mol_type = other DNA
taatacgactcactaatggggaattgtgagcg

SEQ ID NO: 3 - DNA, 32 bp, synthetic construct
  misc_feature 1..32: note = TM2 promoter
  source 1..32: mol_type = other DNA
taatacgactcactcgaggggaattgtgagcg

SEQ ID NO: 4 - DNA, 32 bp, synthetic construct
  misc_feature 1..32: note = TM3 promoter
  source 1..32: mol_type = other DNA
taatacgactcactataaaggaattgtgagcg